European Patent Application EP 4 198 054 A1, published June 21, 2023. Title: ANTI-HMMW ANTIBODY, COMPOSITION COMPRISING SAME, AND NUCLEIC ACID MOLECULE ENCODING SAME, AND USE THEREOF. Applicant: NANJING ANJI BIOLOGICAL TECHNOLOGY CO., LTD. The sequence listing filed with the application follows.

SEQUENCE LISTING (82 sequences)

SEQ ID NO: 1 - protein, 8 aa, synthetic construct
GFTFSNYW

SEQ ID NO: 2 - protein, 10 aa, synthetic construct
IKLKSNNYAT

SEQ ID NO: 3 - protein, 9 aa, synthetic construct
CITEIFDYW

SEQ ID NO: 4 - protein, 9 aa, synthetic construct
TGAVTTSNY

SEQ ID NO: 5 - skipped

SEQ ID NO: 6 - protein, 9 aa, synthetic construct
ALWFLNHWV

SEQ ID NO: 7 - protein, 161 aa, synthetic construct
FLFSDKHRNRTFTMYLGLNCVFIVFLLKGVQSEVKLEESGGGLVQPGGSMKFSCVASGFTFSNYWMNWVRQSPERGLEWVAEIKLKSNNYATLYAESVKGRFTISRDDSKSSVYLQVNNLRAEDTGIYYCITEIFDYWGQGTTLTVSSAKTTPPSVYPLAP

SEQ ID NO: 8 - protein, 133 aa, synthetic construct
SLILSLLALSSGAISQAVVTQESALTTSPGETVTLTCRSSTGAVTTSNYATWVQEKPDHLFTGLIVGANNRAPGVPARFSGSLIGDKAALTITGAQTEDEAIYFCALWFLNHWVFGGGTKLTVLGQPKSSPSV

SEQ ID NO: 9 - DNA, 483 bp, synthetic construct
  source 1..483: mol_type = other DNA
tttctcttcagtgacaaacacagaaatagaacattcaccatgtacttgggactgaactgtgtattcatagtttttctcttaaaaggtgtccagagtgaagtgaagcttgaggagtctggaggaggcttggtgcaacctggaggatccatgaaattctcctgtgttgcctctggattcactttcagtaactactggatgaactgggtccgccaatctccagaaagggggcttgagtgggttgctgaaattaaattgaaatctaataattatgcaacactttatgcggagtctgtgaaagggaggttcaccatctcaagagatgattccaaaagtagtgtctacctacaagtgaacaacttaagagctgaagacactggcatttattactgcatcactgagatttttgactactggggccaaggcaccactctcacagtctcctcagccaaaacgacacccccatctgtctatccactggcccct

SEQ ID NO: 10 - DNA, 399 bp, synthetic construct
  source 1..399: mol_type = other DNA
tcacttatactctctctcctggctctcagctcaggggccatttcccaggctgttgtgactcaggaatctgcactcaccacatcacctggtgaaacagtcacactcacttgtcgctcaagtactggggctgttacaactagtaactatgccacctgggtccaagaaaaaccagatcatttattcactggtctaatagttggtgccaacaaccgagctccaggtgttcctgccagattctcaggctccctgattggagacaaggctgccctcaccatcaccggggcacagactgaggatgaggcaatatatttctgtgctctatggttcctcaaccattgggtgttcggtggaggaaccaaactgactgtcctaggccagcccaagtcttcgccatcagtc

SEQ ID NO: 11 - protein, 8 aa, synthetic construct
GFTFSNYW

SEQ ID NO: 12 - protein, 10 aa, synthetic construct
IRLKSNNYAT

SEQ ID NO: 13 - protein, 9 aa, synthetic construct
CTTEAVDYW

SEQ ID NO: 14 - protein, 16 aa, synthetic construct
RSSKSLLHSNGITYLY

SEQ ID NO: 15 - protein, 7 aa, synthetic construct
QMSNLAS

SEQ ID NO: 16 - protein, 10 aa, synthetic construct
CAQNLELPTF

SEQ ID NO: 17 - protein, 168 aa, synthetic construct
TTLDSQVFLFSDKHRNRTFTMYLGLNCVFIVFLLKGVQSEVKLEESGGGLVQPGGSMKVSCVGSGFTFSNYWMNWVRQSPEKGLEWVAEIRLKSNNYATHYAESVKGRFTISRDDSKRSVYLQMNNLRVEDTGIYYCTTEAVDYWGQGTSVTVSSAKTTPPSVYPLAP

SEQ ID NO: 18 - protein, 148 aa, synthetic construct
DSPYQVRRMRFSAQLLGLLVLWIPGSTADIVMTQAAFSNPVTLGTSASISCRSSKSLLHSNGITYLYWYLQKPGQSPQLLIYQMSNLASGVPDRFSSSGSGTDFTLRISRVEAEDVGVYYCAQNLELPTFGGGTKLEIKRADAAPTVS

SEQ ID NO: 19 - DNA, 504 bp, synthetic construct
  source 1..504: mol_type = other DNA
acaaccctggactcacaagtctttctcttcagtgacaaacacagaaatagaacattcaccatgtacttgggactgaactgtgtattcatagtttttctcttaaaaggtgtccagagtgaggtgaagcttgaggagtctggaggaggcttggtgcaacctggaggatccatgaaagtctcctgtgttggctctggattcactttcagtaactactggatgaactgggtccgccagtctccagagaaggggcttgagtgggttgctgaaattagattgaaatctaataattatgcaacacattatgcggagtctgtgaaagggaggttcaccatctcaagagatgattccaaaaggagtgtatacctgcaaatgaacaacttaagagttgaagacactggcatttattactgtacgactgaggctgtggactactggggtcaaggaacctcagtcaccgtctcctcagccaaaacgacacccccatctgtctatccactggcccct

SEQ ID NO: 20 - DNA, 444 bp, synthetic construct
  source 1..444: mol_type = other DNA
gactcaccatatcaagttcgcagaatgaggttctctgctcagcttctggggctgcttgtgctctggatccctggatccactgcagatattgtgatgacgcaggctgcattctccaatccagtcactcttggaacatcagcttccatctcctgcaggtctagtaagagtctcctacatagtaatggcatcacttatttgtattggtatctgcagaagccaggccagtctcctcagctcctgatttatcagatgtccaaccttgcctcaggagtcccagacaggttcagtagcagtgggtcaggaactgatttcacactgagaatcagcagagtggaggctgaggatgtgggtgtttattactgtgctcaaaatttagaacttcctacgttcggtggaggcaccaagctggaaatcaaacgggctgatgctgcaccaactgtatcc

SEQ ID NO: 21 - protein, 8 aa, synthetic construct
GFTFSDYW

SEQ ID NO: 22 - protein, 10 aa, synthetic construct
IRLKSDNYAT

SEQ ID NO: 23 - protein, 7 aa, synthetic construct
SVETMDF

SEQ ID NO: 24 - protein, 9 aa, synthetic construct
IGAVTTNNY

SEQ ID NO: 25 - skipped

SEQ ID NO: 26 - protein, 9 aa, synthetic construct
ALWYSNHWV

SEQ ID NO: 27 - protein, 116 aa, synthetic construct
EVKLEESGGGLVQPGGSMKLSCVASGFTFSDYWMNWVRQSPEKGLEWLTEIRLKSDNYATHYAESVKGKFTISRDDSKSTVYLQMNNLRAEDTGIYYCSVETMDFWGQGTSVTVSS

SEQ ID NO: 28 - protein, 109 aa, synthetic construct
QAVVTQESALTTSPGETVTLTCRSSIGAVTTNNYANWVQEKPDRLFTGLIRGTNNRVPGVPARFSGSLIGDKAALTITGAQTEDEAIYFCALWYSNHWVFGGGTKLTVL

SEQ ID NO: 29 - DNA, 348 bp, synthetic construct
  source 1..348: mol_type = other DNA
gaagtgaaacttgaggagtctggaggaggcttggtgcaacctggaggatccatgaaactctcctgtgttgcctctggtttcactttcagtgactactggatgaactgggtccgccagtctccagaaaagggtcttgagtggcttactgaaattagattgaaatctgataattatgcaacacattatgcggagtctgtgaaagggaagttcaccatctcaagagatgattccaaaagtactgtctacctgcaaatgaacaacttaagagctgaagacactggcatttattactgttctgtggaaactatggacttctggggtcaaggaacctcagtcaccgtctcctca

SEQ ID NO: 30 - DNA, 327 bp, synthetic construct
  source 1..327: mol_type = other DNA
caggctgttgtgactcaggaatctgcactcaccacatcacctggtgaaacagtcacactcacttgtcgctcaagtattggggctgttacaactaataattatgccaactgggtccaagaaaaaccagatcgtttattcactggtctaattcgtggtaccaacaaccgagttccaggtgttcctgccagattctcaggctccctgattggagacaaggctgccctcaccatcacaggggcacagactgaggatgaggcaatatatttctgtgctctatggtacagcaaccattgggtgttcggtggaggaaccaaactgactgtcctc

SEQ ID NO: 31 - protein, 8 aa, synthetic construct
GFTFSDYW

SEQ ID NO: 32 - protein, 10 aa, synthetic construct
IRLKSNNYLT

SEQ ID NO: 33 - protein, 7 aa, synthetic construct
SVETMDY

SEQ ID NO: 34 - protein, 9 aa, synthetic construct
TGAVTTSNY

SEQ ID NO: 35 - skipped

SEQ ID NO: 36 - protein, 9 aa, synthetic construct
ALWYSNHWV

SEQ ID NO: 37 - protein, 116 aa, synthetic construct
EVKLEESGGGLVQPGGSMKLSCVASGFTFSDYWMNWVRQSPEKGLEWLTEIRLKSNNYLTHYAESVKGRFTISRDDSKSSVYLQMNNLRAEDTGIYYCSVETMDYWGQGISVTVSS

SEQ ID NO: 38 - protein, 109 aa, synthetic construct
QAVVTQESALTTSSGETVTLTCRSSTGAVTTSNYANWVQEKPDHLFTGLIRGTNNRAPGVPARFSGSLIGDKAALTITGAQTEDEAIYFCALWYSNHWVFGGGTKLTVL

SEQ ID NO: 39 - DNA, 348 bp, synthetic construct
  source 1..348: mol_type = other DNA
gaagtgaaacttgaggagtctggaggaggcttggtgcaacctggaggatccatgaaactctcctgtgttgcctctggattcactttcagtgactactggatgaactgggtccgccagtctccagagaagggtcttgagtggcttactgaaattagattgaaatctaataattatttaacacattatgcggagtctgtgaaagggaggttcaccatctcaagagatgattccaaaagtagtgtctacctacaaatgaacaacttaagagctgaagacactggcatttattactgttctgtggaaactatggactattggggtcaaggaatttcagtcaccgtctcctca

SEQ ID NO: 40 - DNA, 327 bp, synthetic construct
  source 1..327: mol_type = other DNA
caggctgttgtgactcaggaatctgcactcaccacatcatctggtgaaacagtcacactcacttgtcgctcaagtactggggctgttacaactagtaactatgccaactgggtccaagaaaaaccagatcatttattcactggtctaatacgtggtaccaacaaccgagctccaggtgttcctgccagattctcaggctccctgattggagacaaggctgccctcaccatcacaggggcacagactgaggatgaggcaatatatttctgtgctctatggtacagcaaccattgggtgttcggtggaggaaccaaactgactgtccta

SEQ ID NO: 41 - protein, 8 aa, synthetic construct
GFTFSNYW

SEQ ID NO: 42 - protein, 10 aa, synthetic construct
IKLKSNNYAT

SEQ ID NO: 43 - protein, 9 aa, synthetic construct
CITEIFDYW

SEQ ID NO: 44 - protein, 9 aa, synthetic construct
TGSVTTSNY

SEQ ID NO: 45 - skipped

SEQ ID NO: 46 - protein, 9 aa, synthetic construct
ALWFIDHWV

SEQ ID NO: 47 - protein, 116 aa, synthetic construct
EVKLEESGGGLVQPGGSMKLSCVVSGFTFSNYWMNWVRQSPERGLEWVAEIKLKSNNYATLYAASVKGRFTISRDDSKSSVYLQVNNLRTEDTGIYYCITEIFDYWGQGTTLTVSS

SEQ ID NO: 48 - protein, 109 aa, synthetic construct
QTVVTQESALTTSPGETVTLTCRSSTGSVTTSNYATWVQEKPDHLFTGLIVGANNRAPGVPARFSGSLIGDKAALTITGAQTEDEAIYFCALWFIDHWVFGGGTKLTVL

SEQ ID NO: 49 - DNA, 348 bp, synthetic construct
  source 1..348: mol_type = other DNA
gaagtgaagcttgaggagtctggaggaggcttggtgcaacctggaggatccatgaaactctcctgtgttgtctctggattcactttcagtaactactggatgaactgggtccgccaatctccagaaagggggcttgagtgggttgctgaaattaaattgaaatctaataattatgcaacactttatgcggcgtctgtgaaagggaggttcaccatctcaagagatgattccaaaagtagtgtctacctgcaagtgaacaacttaagaactgaagacactggcatttattactgcatcactgagatttttgactattggggccaaggcaccactctcacagtctcctca

SEQ ID NO: 50 - DNA, 327 bp, synthetic construct
  source 1..327: mol_type = other DNA
cagactgttgtgactcaggaatctgcactcaccacatcacctggtgaaacagtcacactcacttgtcgctcaagtactgggtctgttacaactagtaactatgccacctgggtccaagaaaaaccagatcatttattcactggtctaatagttggtgccaacaaccgagctccaggtgttcctgccagattctcaggctccctgattggagacaaggctgccctcaccatcaccggggcacagactgaggatgaggcaatatatttctgtgctctatggttcatcgaccattgggtgttcggtggaggaaccaaactgactgtccta

SEQ ID NO: 51 - protein, 8 aa, synthetic construct
GFTFSNYW

SEQ ID NO: 52 - protein, 10 aa, synthetic construct
IRLKSNNYAT

SEQ ID NO: 53 - protein, 7 aa, synthetic construct
TLEAVDY

SEQ ID NO: 54 - protein, 11 aa, synthetic construct
KSLLHSDGITY

SEQ ID NO: 55 - protein, 7 aa, synthetic construct
QMSNLAS

SEQ ID NO: 56 - protein, 10 aa, synthetic construct
CAQNLELPTF

SEQ ID NO: 57 - protein, 116 aa, synthetic construct
EVKLEESGGGLVQPGGSMKLSCVASGFTFSNYWMNWVRQSPEKGLEWVAEIRLKSNNYATHYAESVTGRFTISRDDSKSSVYLQMNNLRAEDTGIYYCTLEAVDYWGQGTSVTVSS

SEQ ID NO: 58 - protein, 111 aa, synthetic construct
DIVMTQAAFSNPVTLGTSASISCRSSKSLLHSDGITYLYWFLQKPGQSPQLLIYQMSNLASGVPDRFSSSGSGTDFTLRISRVEAEDVGVYYCAQNLELPTFGGGTKLEIK

SEQ ID NO: 59 - DNA, 348 bp, synthetic construct
  source 1..348: mol_type = other DNA
gaagtgaagcttgaggagtctggaggaggcttggtgcaacctggaggatccatgaaactctcctgtgttgcctctggattcactttcagtaactactggatgaactgggtccgccagtctccagagaaggggcttgagtgggttgctgaaattagattaaaatctaataattatgcaacacattatgcggagtctgtgacagggaggttcaccatctcaagagatgattccaaaagtagtgtctacctgcaaatgaacaacttaagagctgaagacactggcatttattactgtacacttgaggctgtggactactggggtcaaggaacctcagtcaccgtctcctca

SEQ ID NO: 60 - DNA, 333 bp, synthetic construct
  source 1..333: mol_type = other DNA
gatattgtgatgacgcaggctgcattctccaatccagtcactcttggaacatcagcttccatctcctgcaggtctagtaagagtctcctacatagtgatggcatcacttatttgtattggtttctacagaagccaggccagtctcctcaactcctgatttatcagatgtccaaccttgcctcaggagtcccagacaggttcagtagcagtgggtcaggaactgatttcacactgagaatcagcagagtggaggctgaggatgtgggtgtttattactgtgctcaaaatctagaacttcctacgttcggtggaggcaccaagctggaaatcaaa

SEQ ID NO: 61 - protein, 8 aa, synthetic construct
GFTFSNYW

SEQ ID NO: 62 - protein, 10 aa, synthetic construct
IQLKSNNYAT

SEQ ID NO: 63 - protein, 7 aa, synthetic construct
TTEIFDF

SEQ ID NO: 64 - protein, 11 aa, synthetic construct
QSLLHSDGKTY

SEQ ID NO: 65 - skipped

SEQ ID NO: 66 - protein, 9 aa, synthetic construct
WQGIHFPHT

SEQ ID NO: 67 - protein, 116 aa, synthetic construct
EVKLEESGGGLVQPGGSKKLSCFASGFTFSNYWMNWVRQSPEKGLEWVAEIQLKSNNYATHYAESVKGRFTISRDDSKSSVYLQMNNLRAEDTGIYYCTTEIFDFWGQGTTLTVSS

SEQ ID NO: 68 - protein, 112 aa, synthetic construct
DVVMTQTPLTLSVTIGQPASISCKSSQSLLHSDGKTYLSWLLQRPGQSPKRLIYLVSKLDSGVPDRFTGSGSGTDFTLKISRVEAEDLGVYYCWQGIHFPHTFGGGTKLEIK

SEQ ID NO: 69 - DNA, 348 bp, synthetic construct
  source 1..348: mol_type = other DNA
gaagtgaagcttgaggagtctggaggaggcttggtgcaacctggaggatccaaaaagctctcctgttttgcctctggattcactttcagtaactactggatgaactgggtccgccagtctcctgagaaggggcttgagtgggttgctgagattcaattgaaatctaataattatgcaacacattatgcggagtctgtgaaagggaggttcaccatctcaagagatgattccaaaagtagtgtctacctgcaaatgaacaacttaagagctgaagacactggcatttattactgtaccactgagatttttgacttctggggccagggcaccactctcacagtctcctca

SEQ ID NO: 70 - DNA, 336 bp, synthetic construct
  source 1..336: mol_type = other DNA
gatgttgtgatgacccagactccactcactttgtcggtcaccattggacaaccagcctccatctcttgcaagtcaagtcagagcctcttacatagtgatggaaagacatatttgagttggttgttacagaggccaggccagtctccaaagcgcctaatctatctggtgtctaaactggactctggagtccctgacaggttcactggcagtggatcagggacagatttcacactgaaaatcagcagagtggaggctgaggatttgggagtttattattgctggcaaggtatacattttcctcacacgttcggaggggggaccaagctggaaataaaa

SEQ ID NO: 71 - protein, 8 aa, synthetic construct
GFTFSNYW

SEQ ID NO: 72 - protein, 10 aa, synthetic construct
IKLKSDIDAT

SEQ ID NO: 73 - protein, 7 aa, synthetic construct
STEIFDY

SEQ ID NO: 74 - protein, 11 aa, synthetic construct
QSLLHSDGKTY

SEQ ID NO: 75 - skipped

SEQ ID NO: 76 - protein, 9 aa, synthetic construct
CQYIHFPHT

SEQ ID NO: 77 - protein, 116 aa, synthetic construct
EVKLEESGGGLVQPGGSMKVSCVASGFTFSNYWMNWVRQSPEKGLEWVAEIKLKSDIDATNYAESVKGRFTISRDDSKSSVSLQMNNLRAEDTGIYYCSTEIFDYWGQGTTLTVSS

SEQ ID NO: 78 - protein, 112 aa, synthetic construct
DVVMTQTPLTLSVTIGQPASISCKSSQSLLHSDGKTYLSWLLQRPGQSPKRLIYLVSKLDSGVPDRFTGSGSGTDFTLKISRVEAEDLGIYYCCQYIHFPHTFGGGTKLEIK

SEQ ID NO: 79 - DNA, 348 bp, synthetic construct
  source 1..348: mol_type = other DNA
gaagtgaagcttgaggagtctggaggaggcttggtgcaacctggaggatccatgaaagtctcctgtgttgcctctggattcactttcagtaattactggatgaattgggtccgccagtctccagagaaggggcttgagtgggttgctgaaattaaattgaaatctgatattgatgcaacaaattatgcggagtctgtgaaagggaggttcaccatctcaagagatgattccaaaagtagtgtctccctgcaaatgaacaacttaagagctgaagacactggcatttattactgttccactgagatttttgactactggggccaaggcaccactctcacagtctcctca

SEQ ID NO: 80 - DNA, 336 bp, synthetic construct
  source 1..336: mol_type = other DNA
gatgttgtgatgacccagactccactcactttgtcggttaccattggacaaccagcctccatctcttgcaagtcaagtcagagcctcttacatagtgatggaaagacatatttgagttggttgttacagaggccaggccagtctccaaagcgcctaatctatctggtgtctaaactggactctggagtccctgacaggttcactggcagtggatcagggacagatttcacactgaaaatcagcagagtggaggctgaggatttgggaatttattattgctgccaatatatacattttcctcacacgttcggaggggggaccaagctggaaataaag

SEQ ID NO: 81 - protein, 51 aa, synthetic construct
MERAGVPGFSPRRSSVEAKMQSTSCSVRKSSTVTAWPAVVLLLSWGQRRGG

SEQ ID NO: 82 - DNA, 156 bp, synthetic construct
  source 1..156: mol_type = other DNA
atggagagagcaggggtgcccgggttctctccgcggcgctcatcggtggaggcgaagatgcagagcaccagctgcagtgtcaggaagagctccacagtcaccgcctggccagccgtcgtgctgttgctgagctggggacagagaagaggcggatga